European Patent Specification EP 3 564 364 B1, published September 25, 2024. Title: PREPARING METHODS FOR PLURIPOTENT STEM CELL DERIVED-NEURONAL PROGENITOR CELL INHIBITING FORMATION OF TERATOMA. Applicant: JEIL PHARMACEUTICAL CO.,LTD. The sequence listing filed with the application follows.

SEQUENCE LISTING (14 sequences)

SEQ ID NO: 1 - DNA, 20 bp, Artificial Sequence
  Gapdh F
accacagtccatgccatcac

SEQ ID NO: 2 - DNA, 19 bp, Artificial Sequence
  Gapdh R
tccaccaccctgttgctgt

SEQ ID NO: 3 - DNA, 22 bp, Artificial Sequence
  04-Oct F
cgttctctttggaaaggtgttc

SEQ ID NO: 4 - DNA, 20 bp, Artificial Sequence
  04-Oct R
acactcggaccacgtctttc

SEQ ID NO: 5 - DNA, 23 bp, Artificial Sequence
  Nanog F
gcgtacgcaaattaaagtccaga

SEQ ID NO: 6 - DNA, 20 bp, Artificial Sequence
  Nanog R
tgctattcttcggccagttg

SEQ ID NO: 7 - DNA, 20 bp, Artificial Sequence
  Pax6 F
ggcaacctacgcaagatggc

SEQ ID NO: 8 - DNA, 20 bp, Artificial Sequence
  Pax6 R
tgagggctgtgtctgttcgg

SEQ ID NO: 9 - DNA, 20 bp, Artificial Sequence
  Sox1 F
caatgcggggaggagaagtc

SEQ ID NO: 10 - DNA, 20 bp, Artificial Sequence
  Sox1 R
ctctggaccaaactgtggcg

SEQ ID NO: 11 - DNA, 21 bp, Artificial Sequence
  Nestin F
cagctggcgcacctcaagatg

SEQ ID NO: 12 - DNA, 23 bp, Artificial Sequence
  Nestin R
agggaagttgggctcaggactgg

SEQ ID NO: 13 - DNA, 22 bp, Artificial Sequence
  NF-M F
gagcgcaaagactacctgaaga

SEQ ID NO: 14 - DNA, 23 bp, Artificial Sequence
  NF-M R
cagcgatttctatatccagagcc